European Patent Specification EP 3 394 277 B1, published November 12, 2025. Title: IMPROVED GRANULAR STARCH CONVERSION ENZYMES AND METHODS. Applicant: Danisco US Inc. The sequence listing filed with the application follows.

SEQUENCE LISTING (34 sequences)

SEQ ID NO: 1 - protein, 599 aa, Trichoderma reesei
SVDDFISTETPIALNNLLCNVGPDGCRAFGTSAGAVIASPSTIDPDYYYMWTRDSALVFKNLIDRFTETYDAGLQRRIEQYITAQVTLQGLSNPSGSLADGSGLGEPKFELTLKPFTGNWGRPQRDGPALRAIALIGYSKWLINNNYQSTVSNVIWPIVRNDLNYVAQYWNQTGFDLWEEVNGSSFFTVANQHRALVEGATLAATLGQSGSAYSSVAPQVLCFLQRFWVSSGGYVDSNINTNEGRTGKDVNSVLTSIHTFDPNLGCDAGTFQPCSDKALSNLKVVVDSFRSIYGVNKGIPAGAAVAIGRYAEDVYYNGNPWYLATFAAAEQLYDAIYVWKKTGSITVTATSLAFFQELVPGVTAGTYSSSSSTFTNIINAVSTYADGFLSEAAKYVPADGSLAEQFDRNSGTPLSALHLTWSYASFLTATARRAGIVPPSWANSSASTIPSTCSGASVVGSYSRPTATSFPPSQTPKPGVPSGTPYTPLPCATPTSVAVTFHELVSTQFGQTVKVAGNAAALGNWSTSAAVALDAVNYADNHPLWIGTVNLEAGDVVEYKYINVGQDGSVTWESDPNHTYTVPAVACVTQVVKEDTWQS

SEQ ID NO: 2 - protein, 619 aa, Aspergillus kawachii
LSAAEWRTQSIYFLLTDRFGRTDNSTTATCNTGDQIYCGGSWQGIINHLDYIQGMGFTAIWISPITEQLPQDTSDGEAYHGYWQQKIYNVNSNFGTADDLKSLSDALHARGMYLMVDVVPNHMGYAGNGNDVDYSVFDPFDSSSYFHPYCLITDWDNLTMVQDCWEGDTIVSLPDLNTTETAVRTIWYDWVADLVSNYSVDGLRIDSVEEVEPDFFPGYQEAAGVYCVGEVDNGNPALDCPYQKYLDGVLNYPIYWQLLYAFESSSGSISNLYNMIKSVASDCSDPTLLGNFIENHDNPRFASYTSDYSQAKNVLSYIFLSDGIPIVYAGEEQHYSGGDVPYNREATWLSGYDTSAELYTWIATTNAIRKLAISADSDYITYANDPIYTDSNTIAMRKGTSGSQIITVLSNKGSSGSSYTLTLSGSGYTSGTKLIEAYTCTSVTVDSNGDIPVPMASGLPRVLLPASVVDSSSLCGGSGNTTTTTTAATSTSKATTSSSSSSAAATTSSSCTATSTTLPITFEELVTTTYGEEVYLSGSISQLGEWDTSDAVKLSADDYTSSNPEWSVTVSLPVGTTFEYKFIKVDEGGSVTWESDPNREYTVPECGSGSGETVVDTWR

SEQ ID NO: 3 - protein, 616 aa, Aspergillus Terreus
APQLAPRATTSLDAWLASETTVALDGILDNVGSSGAYAKSAKSGIVIASPSTSDPDYYYTWTRDAALTVKALIDLFRNGETSLQTVIMEYISSQAYLQTVSNPSGSLSTGGLAEPKYYVDETAYTGSWGRPQRDGPALRATAMIDFGNWLIDNGYSTYASSIVWPIVRNDLSYVAQYWNQTGYDLWEEVNGSSFFTIAVQHRALVEGSTFASKVGASCSWCDSQAPQVLCFLQRFWTGSYIMANFGGGRSGKDANTVLGSIHTFDPNAGCDDTTFQPCSPRALANHKVYTDSFRSIYSINSGISSGKAVAVGRYPEDSYYNGNPWFLTTLAAAEQLYDAIYQWQKIGSITITDVSLAFFKDLYSSAAVGTYASSSSAFTSIVSAVKTYADGYMSIVQTHAMTNGSLSEQFGKSDGFSLSARDLTWSYAALLTANLRRNSVVPPSWGETTATSVPSVCSATSATGTYSTATNTAWPSTLTSGTGATTTTSKATSSSTTTTSSASSTTVECVVPTAVAVTFDEVATTTYGENVYVVGSISQLGSWDTSKAVALSASKYTSSNNLWYVTVTLPAGTTFQYKFIRVSSSGSVTWESDPNRSYTVPSACGTSTAVVNTTWR

SEQ ID NO: 4 - protein, 612 aa, Aspergillus fumigatus
APQLSARATGSLDSWLGTETTVALNGILANIGADGAYAKSAKPGIIIASPSTSEPDYYYTWTRDAALVTKVLVDLFRNGNLGLQKVITEYVNSQAYLQTVSNPSGGLASGGLAEPKYNVDMTAFTGAWGRPQRDGPALRATALIDFGNWLIDNGYSSYAVNNIWPIVRNDLSYVSQYWSQSGFDLWEEVNSMSFFTVAVQHRALVEGSTFAKRVGASCSWCDSQAPQILCYMQSFWTGSYINANTGGGRSGKDANTVLASIHTFDPEAGCDDTTFQPCSPRALANHKVYTDSFRSVYAINSGIPQGAAVSAGRYPEDVYYNGNPWFLTTLAAAEQLYDAIYQWKKIGSISITSTSLAFFKDIYSSAAVGTYASSTSTFTDIINAVKTYADGYVSIVQAHAMNNGSLSEQFDKSSGLSLSARDLTWSYAAFLTANMRRNGVVPAPWGAASANSVPSSCSMGSATGTYSTATATSWPSTLTSGSPGSTTTVGTTTSTTSGTAAETACATPTAVAVTFNEIATTTYGENVYIVGSISELGNWDTSKAVALSASKYTSSNNLWYVSVTLPAGTTFEYKYIRKESDGSIVWESDPNRSYTVPAACGVSTATENDTWQ

SEQ ID NO: 5 - protein, 608 aa, Neosartorya fischeri
APQLSPRATGSLDSWLATESTVSLNGILANIGADGAYAKSAKPGIIIASPSTSDPDYYYTWTRDAALVTKVLVDLFRNGNLGLQKVITEYVNSQAYLQTVSTPSGGLSSGGLAEPKYNVDMTAFTGAWGRPQRDGPALRATALIDFGNWLIDNGYSSYAVNNIWPIVRNDLSYVSQYWSQSGFDLWEEVNSMSFFTVAVQHRALVEGSTFAKRVGASCSWCDSQAPQILCYMQSFWTGSYINANTGGGRSGKDANTVLASIHTFDPEAGCDDTTFQPCSPRALANHKVYTDSFRSVYAINSGIPQGVAVSAGRYPEDVYYNGNPWFLTTLAAAEQLYDAIYQWKKIGSISITSTSLAFFKDIYSSVAVGTYASSSSTFTAIIDAVKTYADGYVSIVEAHAMTNGSLSEQFDKSSGMSLSARDLTWSYAALLTANMRRNGVVPAPWGAASANSVPSSCSMGSATGTYSTATATSWPSTLTSGSPSDTTSGTTPGTTTTTSACTTPTSVAVTFDEIATTTYGENVYIIGSISQLGSWDTSKAVPLSSSKYTSSNNLWYVTINLPAGTTFEYKYIRKESDGSIEWESDPNRSYTVPSACGVSTATEKDTWR

SEQ ID NO: 6 - protein, 612 aa, Neosartorya fumigata
APQLSARATGSLDSWLGTETTVALNGILANIGADGAYAKSAKPGIIIASPSTSEPDYYYTWTRDAALVTKVLVDLFRNGNLGLQKVITEYVNSQAYLQTVSNPSGGLASGGLAEPKYNVDMTAFTGAWGRPQRDGPALRATALIDFGNWLIDNGYSSYAVNNIWPIVRNDLSYVSQYWSQSGFDLWEEVNSMSFFTVAVQHRALVEGSTFAKRVGASCSWCDSQAPQILCYMQSFWTGSYINANTGGGRSGKDANTVLASIHTFDPEAGCDDTTFQPCSPRALANHKVYTDSFRSVYAINSGIPQGAAVSAGRYPEDVYYNGNPWFLTTLAAAEQLYDAIYQWKKIGSISITSTSLAFFKDIYSSAAVGTYASSTSTFTDIINAVKTYADGYVSIVQAHAMNNGSLSEQFDKSSGLSLSARDLTWSYAAFLTANMRRNGVVPAPWGAASANSVPSSCSMGSATGTYSTATATSWPSTLTSGSPGSTTTVGTTTSTTSGTATETACATPTAVAVTFNEIATTTYGENVYIVGSISELGNWDTSKAVALSASKYTSSNNLWYVSVTLPAGTTFEYKYIRKESDGSIVWESDPNRSYTVPAACGVSTATENDTWR

SEQ ID NO: 7 - protein, 618 aa, Penicillium marneffei
APQFSPRATVGLDAWLASETTFSLNGILANIGSSGAYSASAKPGVVIASPSTNNPNYYYTWTRDSALTLKVLIDLFGNGNLSLQTVIEEYINAQAYLQTVSNPSGDLSSGAGLAEPKYNVDMSPFTGGWGRPQRDGPALRAIALIEFGNWLIDNGYSSYAVNNIWPIVRNDLSYVSQYWSQSGFDLWEEVNSMSFFTVANQHRALVQGSTFAARVGASCSWCDSQAPQILCYMQTFWTGSYINANTGGGRSGKDSNTVLTTIHTFDPEATCDDVTFQPCSPRALANHKVYTDSFRSIYGVNSGIAQGVAVSVGRYPEDSYYGGNPWFLSNLAAAEQLYDAIYQWNKIGSITITSTSLAFFKDVYSSAAVGTYASGSTAFTSIISAVKTYADGYVSIVQGHAAANGSLSEQFDRNSGVEISARDLTWSYAALLTANLRRNGVMPPSWGAASANSVPSSCSMGSATGTYSTPTATAWPSTLTSATGIPVTTSATASVTKATSATSTTTSATTCTTPTSVAVTFDEIATTTYGENVFIVGSISQLGSWDTSKAIALSASQYTSSNHLWFATLSLPAGTTFQYKYIRKESNGSIVWESDPNRSYTVPSGCGVSTATENDTWR

SEQ ID NO: 8 - protein, 617 aa, Talaromyces stipitatus
APGLSPRASTSLDAWLATETTVSLSGILANIGADGAYSKSAKPGVVIASPSTDNPNYYYTWTRDSALTLKVLIDLFRNGNLGLQTVIEEYVNAQAYLQTVSNPSGDLSSGAGLAEPKFNVDMSAFTGSWGRPQRDGPALRAIALIDFGNWLIENGYTSLAANNIWPIVRNDLSYVAQYWSQSGFDLWEEVNSMSFFTVANQHRSLVEGSTFAAKVGASCSWCDSQAPQILCYMQTFWTGSYMNANTGGGRSGKDANTVLTSIATFDPEATCDDVTFQPCSPRALANHKVYTDSFRSVYGLNSGIAEGVAVAVGRYPEDSYYNGNPWFLSNLAAAEQLYDAIYQWNKIGSITITSTSLAFFKDVYSSAAVGTYASGSSAFTSIINAVKTYADGYISVVQSHAMNNGSLSEQFDKNTGAELSARDLTWSYAALLTANMRRNGVVPPSWGAASATSIPSSCTTGSAIGTYSTPTATSWPSTLTSGTGSPGSTTSATGSVSTSVSATTTSAGSCTTPTSVAVTFDEIATTSYGENVYIVGSISQLGSWNTANAIALSASKYTTSNNLWYVTINLPAGTTFQYKYIRKESDGTVKWESDPNRSYTVPSACGVSTATENDTWR

SEQ ID NO: 9 - protein, 560 aa, Metarhizium acridum
HRDDLHGFITKQKSISLHGVLANIGSDGSRAQGAAAGAVVASPSKSDPDYWYTWSRDSALTFKVLIELFIGGKKSLQPKIEQYITAQAHLQGVSNPSGGPDTGGLGEPKFHVNLTAFTGSWGRPQRDGPPLRATALTIYANWLIANGGQAEAANTVWPIIAKDLSYTVQYWNRTGFDLWEEINGSSFFTLSASFRALVEGATLAKALGKQCPDCETNAPRILCFLQSFWANGYIDSNINVNDGRTGKDVNSIISSIHTFDPAAACTDATFQPCSSRALANHKAVVDSFRTIYTVNKGRRPGRAAAVGRYSEDVYYNGNPWYLATMAAAEQMYAAVYQWREIGSITVDATSLPFFSDLIPNIAAGTYAKNSATFTSIIKAATAYGDDFVRVVKQYTPADGSLAEQYDRETGSPKSAVHLTWSYASFVGAVERRSGIVPPSWGEPNSNTVPKVCEAPPSCDSTMTFNVKVTTVPGESIYVVGSITELKNWSPADAVPLDASQYTPSNPLWSAKVTIPAGTNFEYKYIKKTSDGTVVWESDPNRSATSSTGCQSNGTLNDQWR

SEQ ID NO: 10 - protein, 556 aa, Schizophyllum commune
QTSAADAYVSAESPIAQAGILANIGPSGSKSHGAASGVIIASPSTSNPDYLYTWTRDAALVSRALVDEFIEGESSLQSVIDSYVSSQQKLQRVDNPSGSYTSGGLGEPKFNIDLTAFTGAWGRPQRDGPALRAITLITYGNHLLSSGNTSYVTDTIWPVVKADLDYVVSYWNQTGFDLWEEVSSSSFFTTAEQHTALRLGATFATAVGASASTYLTQADNVLCFLQSYWNSNGGYATANTGGGRSGIDANTVLTSIHTFDIEAGCDSVTFQPCSDRALSNLKVYVDSFRGLYSINPTGATDPILTGRYKEDVYYNGNPWYLTTFAVAEQLYDALNTWDKLGSLDVTSTSLAFFKQFDSSITAGTYASSTSEYATLTSAIRNWADGFLEVLADFTPADGGLTEQIDKSSGNPTSAADLTWSYASAITAFKARGGAIPASWGAAGLTVPATCSTGGGGGSGGDTVAVTLNVQATTVYGENIYVTGSVNQLANWSPDNAIALNADNYPTWSVTVNLPANTQIEYKYIRKNNGQVTWESDPNRSITTSASGSFTQNDTWR

SEQ ID NO: 11 - protein, 627 aa, Trichoderma atroviridis
VPRLRESRHEFDIVKRSASSFLETEVPIALADLLCNIGSAGSCAAGANSGIVIASPSKTNPDYFYTWTRDSALVFKCIVDTFVNSYSASLQTEIENYINAQAIVQGISNPSGSLSNSGTGLGEPKFNVDETAFTGAWGRPQRDGPALRAIALITYSKWLINNGYQSTANSIVWPIIQNDISYVAQYWNQTGFDLWEEVNGSSFFTVANQHRALVEASALATSLGKSLPNASSQAAQALCFLQSFWSSSQGYIVANINQNNGRSGKDANTLLGSIHTFDPEGNCDASTFQPCSDRTLANHKVVVDSFRSIYTINNGIPAGTAAAVGRYPEDSYQGGNPWYLNTLAAAELLYDALYQWKRIGAITVTSTSLAFFKDLDSSITVGTYSSSSSTYTTLYNAVSNYADGFVNNVATYAPSNGSLAEQYNRNNGQPLSAYDLTWSYAALLTAAARRSGVVPYSWGETSASSVPSVCSYTSAVGSYSSASTGSWPPNQTPTDGSGSTTSKSTSVTVSSTSTSASSTAVATSPVTVTFDEIVTTIFGQTIKIAGNVPVLGNWNTNNAVALSADGYTSSNHLWNVGISFAPGTVIQYKYINVASNGDVTWEADPNHTYTVPATGATAVTVNNSWQS

SEQ ID NO: 12 - protein, 561 aa, Bjerkandera adusta
QSSTVDAFIASESPIARTGLLANIGADGSKASGAKSGIVIASPSKSNPDYFYTWTRDAALVFKAIIDRYTSGEDTATRRQIDEYVSGQALLQQVSNPSGTVSTGGLAEPKYNVDMSAFTGGWGRPQRDGPALRATAIIAYANWLVANGNTSYVTSTLWPVLKLDLDYVRDNWNQTGFDLWEEINSSSFFTTAVQHRALREGNALAAKIGQTVSGYTTQADNVLCFLQSYWNPSGGFATSNTGGGRSGKDANSVLTSIHTFDAAAGCDALTFQPCSDRALSNHKVYVDSFRSIYSVNSGIASNAAVATGRYPEDSYYGGNPWYLTTLAAAEQLYDALTVWDAQGSLNVTSVSLAFFQQFAPTVTAGTYPASSATYGTLTAAIRAYADGFVAVVAKYTPSNGGLAEQYTRAGGTPTSAADLTWSYAAALTAFSAREGFTPASWGAKGLTAPAACNTNSGGGSGGGSGNTVAVTFNVQATTVWGENIYLTGSVDALQNWSPDNALLLSSANYPTWSITVNLPPSTAIQYKYIRKNNGAVTWESDPNMSITTPGSGSATLSDTWR

SEQ ID NO: 13 - protein, 558 aa, unknown
  Ganoderma spp.
QSSADAYVASEASIAKAGLLANIGANGSKSEGAKAGIVVASPSTSNPDYLYTWTRDSSLVFKTVIDQFTTGEDTSLRGLIDEFTAAQSILQQTSNPSGSVSTGGLGEPKFNVDETAFTGAWGRPQRDGPALRATAIITYANWLLANGNGTSYVQNTLWPIIKLDLDYVENNWNQSTFDLWEEVNSSSFFTTAVQHRALREGVALASAIGQTSVVSGYSAQADNLLCFLQSYWNSGSGFVTANTGGGRSGRDANTVLTSIHTFDVEAGCDAVTFQPCSDKALSNLKVYVDAFRSIYGINSGIASNAAVATGRYPEDSYYNGNPWYLAVFAVAEQLYDALITWDELGSLNVTSTSLAFFQQFDSSVTAGTYDSSSSTYSTLTSGIKGFADGFLEVNSKYTPSTGALSEQFDKSSGSQLSASDLTWSYAAALTAFAARSGKTYASWGAAGLITTCGGSGGGGGGSGTVSVTFNVQATTVFGENIYITGSVDALQNWSPDNALILSAANYPIWSITVSLPASTVIEYKYIRKFNGQVTWESDPNDSITTPASGSYIENDTWR

SEQ ID NO: 14 - protein, 562 aa, Termetes versicolor
QSSVADAYVASESSIAKAGVLANIGPSGSKSQGAKAGIVVASPSTTNPDYLFTWTRDTSLVFKALIDQLTSGEDPSLRGLVDMFTSSQAALQQVSNPSGTVSTGGLGEPKFNIDESAFTGAWGRPQRDGPALRSTAFISYANWLLDNGNTTYVTQTLWPVIKLDLDYVEANWNQTGFDLWEEVNSSSFFTTAVQHRALREGAAFATRIGQTSVVSGYTTQAANVLCFLQSYWNPSGGFVTANTGGGRSGRDANTVLTSIHTFDPAAGCDATTFQPCSDKALSNLKVYVDAFRSIYTINSGIAANAAVATGRYPEDSYQGGNPWYLATIAVAEQLYDALIVWDQLGSINVTTTSLPFFQQFSSTVTTGTFASTSATYTTLTTAVRNFADGFIAVNAQFTPSNGGLAEQFSRSNGQPVSAVDLTWSYAATLTAFHARAGLTYPGWGAAGLTVPAVCSTSGSGSGGGGAGTVAVTFNVQATTFFGENIYITGSVDALQNWSPDNALLLSSANYPIWSITVNLPASTSVQYKFIRKAPGELIWESDPNNQITTPASGTFTQSDTFR

SEQ ID NO: 15 - protein, 563 aa, Hypholoma sublateritium
QSSAVSSYLATESVIAKAGLLANIGPSGSKASGAVSGVVVAAPSTNPDYIFTWTRDSALVFKAIIDSFARGEDATLRTSIDQYVAAQKIQQQVSNPSGTVSSGGLGEPKFNVDLSAFTGAWGRPQRDGPALRATALISYGNSLISASNTSYVLANIWPLVKLDLDYVAANWNQTGFDLWEEVNSSSFFTTAVQHRALRQGAAFATALGQTASVAGYTTQAANVLCFLQSYWNPSQGYITANTGGGRSGKDANTALASIHTFDPTAGCDAATFQPCSDKALSSLKVYVDSFRSIYTVNSAVASPGAVATGRYPEDSYFGGNPWYLATMAVAEQLYDALIVWKAQGSLNVTSTSLAFFQQFSSAVTVGTYASTTATFTTLTTAIANQADGFVAIVQEFTPSTGSLSEQYSRSNGAQLSANDLTWSYASILTAVTARNGLAGDNWGAAGLVVPSSCSTSGTGSSSGGGSSGTVAVTFKVTATTTFGENIYLTGSDDALEDWSPTSTLILSAATYPVWSITVNLPASTALQYKYIRIFNGVTTWESDPNNAFTTVASGTQTLTDTWR

SEQ ID NO: 16 - protein, 559 aa, Fomitiporia mediterranea
QTAVDSYVATESPIAKTNLLANIGASGSKSQGAKPGIVIASPSTTNPNYLFTWTRDSSLVFKTIIDQYTNGQDTSLRTLIDEFVSAEATLQQVSNPSGTVSTGGLGEPKFNIDETAFTGAWGRPQRDGPALRATAIINYANYLLANDNSSFVTNTLWPILQLDLDYVAQDWNQTTFDLWEEVDSTSFFTAAVQHRSLREGATLATKIGQTSVVSGYTTQAENILCFMQSFWNAGGNFMTANTGGGRSGKDANTVLASIHTFDSSAGCDAATFQPCSDRALANLKTYVDAFRSIYSINSGIASNAAVATGRYPEDVYFNGNPWYLTTLSVAEQLYDAITVWNAQGSLNVTSVSQPFFALFQSDIAVGTYASSSSTFTSLLSSIKSFADGFVSVVAKYTPSNGGLSEQYSKSDGTPTSAVDLTWSYAAALTAFAARDGFVPASWGAAGLTVPSTCSTSGSGPGSGGTVAVTFNVQATTVFGENIYITGSVDALQNWSPDNAIILSAANYPTWSVTINLPASTTIQYKYIRKFNGAVTWESDPNMQITTPSGGTFIENDVWR

SEQ ID NO: 17 - protein, 562 aa, Punctularia strigosozonata
QTASAAAYATTEAPIAKAGVLANIGPSGSKSQGAKAGIVIASPSTSNPDYLYTWTRDSSLVFKALIDQYTSGIDTTLRGAIDNFFNAEKILQQVSNPSGTVSTGGLGEPKFNIDETAFTGAWGRPQRDGPALRATALITYANYLYSTGNTTFVSNTLWPVIKLDLDYAANNWNQTTFDLWEEVSSSSFFTTAVQHRSLREGATLATKLGVTSSASTYTSAASSLLCFLQSYWNPAGGYITANTGGGRSGKDANTVLTSIHTFDPAAGCDAVTFQPCSDKALSNLKVYVDSFRSIYGINSGIASNAAVATGRYPEDTYYNGNPWYLTTLAVAEQLYDALIVWNARGSLNVTSTSLAFFQQFSSSVTTGTYPSTSTTFTTLTSAVKTFADGFVAVVAKYTPSSGALSEQFDKSSGSQLSAADLTWSYAAALTAFEARNGTTFASWGAAGLTTSCSSSGSGSGGGSGSSGSVPVNFQETATTVYGENIFIVGSISPLGNWDPNSAIALSAANYPNWQVSISLPASTTFQYKYIRKYNGAVTWESDPNRSFTTPSSGSYNENDTWR

SEQ ID NO: 18 - protein, 554 aa, Phlebia brevispora Nakasone
QTNVNSYVASESAFAKAGLLANIGPSGSKSSGADPGIVIASPSTTNPDYLYTWVRDSSLVFKVLIDQYTTGVDTSLRTLIDEFVSAEAILQQVTNPSGSVTTGGLGEPKFNIDETAFTGSWGRPQRDGPALRSTAIITYANWLLDNGNTSYVTETLWPVLELDLNYVMNNWNQSTYDLWEEIDSSSFWTTAVQHRALRQGSALATRIGQTSMVSGYNTQAANVLCFLQSFWNPSGNYVTANTGGGRSGIDANTVLTSIHTFDPSAGCDATTFQPCSDKALANLKVYTDSFRSIYSVNTGIASNAAVATGRYPEDVYMGGNPWYLATMAAAEQLYDALSVWESQGSLTVTPTSLAFFQMFDSGVQAGTYASSSSTFSSLTSAIQSLADGFVAIHAEYTPSDGSLSEQFSRSNGSPTSAADLTWSYAAALTGFAARNGTQVASWGAAGLTVPATCQGSPGPTVSVTFNVDATTVWGENIYITGSVDALENWSTTTALLLSSANYPIWSITVSLPANTNIQYKYIRIDNGAVTWESDPNNSLTTPASGSYTVNDTWR

SEQ ID NO: 19 - protein, 621 aa, Sarocladium zeae
RPGPAKVQLSTRAVGDFINSETPIALEQLLCNIGANGCNSAGVSSGLVIASPSKQDPDYWYTWTRDSALVFKSIVDRFTNSYDAGLQRHITDYIVAQARLQGVSNPSGGFSDGSGLAEPKYNVDGSAFTGAWGRPQRDGPALRAIAIMSYGEWLLDNSYTDTAKNIVWPVVRNDLEYVAQYWNQTGFDLWEEVRGSSFFTIASQHQALVQGYRFAARVGASGAHYQATAPSVLCFLQSFWNPSKGYIDSNINVNDGRTGLDANSILASIHTFDASIGCDSTTFQPCSDKALSNLKAVVDSFRFYNINNGIPKGTALAVGRYAEDVYYNGNPWYLNTLAAAEQLYDAVYVWKQQGSVTVTATSRAFFADLIPNIAVGTYQSGSSTYNSIIQAVSQYGDGFVNVVATYAQSNGSLAEQFSKQDGTPLSARDLTWSYASFLTAAARRAGVIPRPWSGGVEALPGTCSAVSFTGSYTSATATNFPASQTPVTGTGTATGTSPPTTSTTAQPPSTTTACAIAPQVTVNFVARVVTNYGDTVKLVGNVDKLGNWNPGSGVVFSASDYQANNPVWKGSVVLSAGQSIQYKYVKVLSDGTVKWEADPNRTYSVPRSCATAVTRSDTWQT

SEQ ID NO: 20 - protein, 611 aa, Penicillium oxalicum
APQLSPRATASLDAWLATETTFSLNGILNNIGASGAYAKSAKNGVVIASPSTSSPNYYYTWSRDSALTLKVLIDLFRNGNLDLQTVIEEYINAQATLQTVSNPSGDLSSGAGLGEPKFNVDLSAFTDGWGRPQRDGPALRAISLIEFGNWLIDNGYSSYAINNVWPIVRNDLSYVAQYWSQTGFDLWEEVNSMSFFTVASQHRSLVEGSAFAKRVGASCSWCDSQAPQILCYMQTFWTGSYMNANTGGGRSGKDANTVLASIHTFDPEATCDDITFQPCSPRALANHKVYTDSFRSVYSINSGIAQGVAVAVGRYPEDSYYNGNPWFLSNLAAAEQLYDAIYQWNKIGSITITSTSLAFFKDIYSSAAVGTYASGSSTFTAIISAVKTYADGYVSIVQAHSYTNGSLSEQYDKSTGLSLSARDLTWSYAALLTANMRRNGVVPPSWGASSANTVPSSCSMGSAAGTYATPTATSWPSTLTSGTPGSTTSTPATSTTSTTSTSACTTPTSVAVTFDEIATTTYGENVYIVGSISQLGSWNTANAIALSASQYTSSKHLWYVTINLPAGTTFQYKYIRKESDGSIVWESDPNRSYTVPATCGTTTATENDTWR

SEQ ID NO: 21 - protein, 617 aa, Aspergillus clavatus
LTPAEWRGQSIYFLITDRFARTDGSTTAPCDLSQRAYCGGSWQGIIKQLDYIQGMGFTAIWITPITEQIPQDTAEGSAFHGYWQKDIYNVNSHFGTADDIRALSKALHDRGMYLMIDVVANHMGYNGPGASTDFSTFTPFNSASYFHSYCPINNYNDQSQVENCWLGDNTVALADLYTQHSDVRNIWYSWIKEIVGNYSADGLRIDTVKHVEKDFWTGYTQAAGVYTVGEVLDGDPAYTCPYQGYVDGVLNYPIYYPLLRAFESSSGSMGDLYNMINSVASDCKDPTVLGSFIENHDNPRFASYTKDMSQAKAVISYVILSDGIPIIYSGQEQHYSGGNDPYNREAIWLSGYSTTSELYKFIATTNKIRQLAISKDSSYLTSRNNPFYTDSNTIAMRKGSGGSQVITVLSNSGSNGGSYTLNLGNSGYSSGANLVEVYTCSSVTVGSDGKIPVPMASGLPRVLVPASWMSGSGLCGSSSTTTLVTATTTPTGSSSSTTLATAVTTPTGSCKTATTVPVVLEESVRTSYGENIFISGSIPQLGSWNPDKAVALSSSQYTSSNPLWAVTLDLPVGTSFEYKFLKKEQNGGVAWENDPNRSYTVPEACAGTSQKVDSSWR

SEQ ID NO: 22 - protein, 587 aa, Aspergillus Terreus
LTPAEWRSQSIYFLLTDRFGRTDNSTTAACDTSDRVYCGGSWQGIINQLDYIQGMGFTAIWITPVTGQFYENTGDGTSYHGYWQQDIYDLNYNYGTAQDLKNLANALHERGMYLMVDVVANHMGYDGAGNTVDYSVFNPFSSSSYFHPYCLISNYDNQTNVEDCWLGDTTVSLPDLDTTSTAVRNIWYDWVADLVANYSIDGLRVDTVKHVEKDFWPGYNSAAGVYCVGEVYSGDPAYTCPYQNYMDGVLNYPIYYQLLYAFESSSGSISDLYNMISSVASSCKDPTLLGNFIENHDNPRFASYTSDYSQAKNVITFIFLSDGIPIVYAGQEQHYSGGSDPANREATWLSGYSTSATLYTWIATTNQIRSLAISKDAGYVQAKNNPFYSDSNTIAMRKGTTAGAQVITVLSNKGASGSSYTLSLSGTGYSAGATLVETYTCTTVTVDSSGNLPVPMTSGLPRVFVPSSWVNGSALCNTECTAATSISVLFEELVTTTYGENIYLSGSISQLGSWNTASAVALSASQYTSSNPEWYVSVTLPVGTSFQYKFIKKGSDGSVVWESDPNRSYTVPAGCEGATVTVADTWR

SEQ ID NO: 23 - protein, 607 aa, Aspergillus fumigatus
LTPAEWRSQSIYFLLTDRFGREDNSTTAACDVTQRLYCGGSWQGIINHLDYIQGMGFTAIWITPVTEQFYENTGDGTSYHGYWQQNIHEVNANYGTAQDLRDLANALHARGMYLMVDVVANHMGYNGAGNSVNYGVFTPFDSATYFHPYCLITDYNNQTAVEDCWLGDTTVSLPDLDTTSTAVRSIWYDWVKGLVANYSIDGLRIDTVKHVEKDFWPGYNDAAGVYCVGEVFSGDPQYTCPYQNYLDGVLNYPIYYQLLYAFQSTSGSISNLYNMISSVASDCADPTLLGNFIENHDNPRFASYTSDYSQAKNVISFMFFSDGIPIVYAGQEQHYSGGADPANREAVWLSGYSTSATLYSWIASTNKIRKLAISKDSAYITSKNNPFYYDSNTLAMRKGSVAGSQVITVLSNKGSSGSSYTLSLSGTGYSAGATLVEMYTCTTLTVDSSGNLAVPMVSGLPRVFVPSSWVSGSGLCGDSISTTATAPSATTSATATRTACAAATAIPILFEELVTTTYGESIYLTGSISQLGNWDTSSAIALSASKYTSSNPEWYVTVTLPVGTSFEYKFVKKGSDGSIAWESDPNRSYTVPTGCAGTTVTVSDTWR

SEQ ID NO: 24 - protein, 609 aa, Neosartorya fischeri
LTPAEWRSQSIYFLLTDRFGREDNSTTAACDVTQRLYCGGSWQGIINHLDYIQGMGFTAIWITPVTQQFYENTGDGTSYHGYWQQNIYEVNSNYGTAQDLRKLADALHARGMYLMVDVVANHMGYDGAGNSVDYSVFTPFDSSTYFHTYCLISDYNNQNNVEDCWLGDTTVSLPDLDTTNTAVRTIWYDWVKGLVANYSIDGLRIDTVKHVEKDFWPDYNDAAGVYCVGEVFSGDPSYTCPYQNYMDGVLNYPIYYQLLYAFQSTSGSISNLYNMISSVDSDCADPTLLGNFIENHDNPRFASYTSDYSQAKNVISFMFFSDGIPIVYAGQEQHYSGGADPANREAVWLSGYSTSATLYSWIASTNKIRKLAISKDSAYITSKNNPFYYDSNTLAMRKGSVAGSQVITVLSNKGSSGSSYTLSLSGTGYSAGATLVEMYTCTTLTVDSSGNLAVPMASGLPRVLVPSSWVSGSGLCGDSISTIATTTTSTTKTTTVATTTACASATALPILFEELVTTTYGETIYLTGSISQLGNWDTSSAIALSASKYTSSNPEWYATVTLPVGTSFQYKFFKKESDGSIVWESDPNRSYTVPAGCAGTTVTVSDTWR

SEQ ID NO: 25 - protein, 603 aa, Talaromyces emersonii
LTPAEWRKQSIYFLLTDRFGRADNSTTAACDVTERIYCGGSWQGIINHLDYIQGMGFTAIWISPVTEQLPQNTGEGEAYHGYWQQEIYTVNSNFGTSDDLLALSKALHDRGMYLMVDVVANHMGYDGDGDSVDYSVFNPFNSSSYFHPYCLITDYSNQTDVEDCWLGDTTVSLPDLNTTETVVRTIWYDWVADLVSNYSIDGLRIDTVKHVEKSFWPGYNSAAGVYCVGEVLDGDPSYTCPYQDYLDGVLNYPIYYQLLYAFESSSGSISNLYNMINSVASECSDPTLLGNFIENHDNPRFASYTSDYSLAKNVIAFIFFSDGIPIVYAGQEQHYNGGNDPYNREATWLSGYSTTAELYTFIATTNAIRSLAISVDSEYLTYKNDPFYYDSNTLAMRKGSDGLQVITVLSNLGADGSSYTLTLSGSGYSSGTELVEAYTCTTVTVDSNGDIPVPMESGLPRVFLPASSFSGSSLCSSSPSPTTTTSTSTSTTSTACTTATAVAVLFEELVTTTYGENVYLSGSISQLGDWNTDDAVALSAANYTSSNPLWYVTVTLPVGTSFEYKFIKKEENGDVEWESDPNRSYTVPTACTGATETIVDTWR

SEQ ID NO: 26 - protein, 612 aa, Penicillium funiculosum
LSAAEWRSQSIYFLLTDRFARTDGSTSAACDLSQRIQAYCGGSWQGIIDHLDYIQGMGFTAVWITPITKQMPQTTSEGTGFHGYWQQDIYSVNPNFGTADDIKALSKAIHDRGMYLMIDVVANHMGYNGAGSSTDFSVFNPFNSASYFHSYCSISDYNNQNQVENCWLGDDTVSLTDLNTQSDQVRTIWYSWVKDLVANYTVDGLRIDTVKHVEKDFWTGYSQAAGVYTLGEVLHGDPAYTCPYQGYVDGVFNYPIYYPLLNAFKSSSGSISSLVSMINSVSSDCKDPTLLGSFIENHDNPRFPSYTSDMSQAKSVIGYVFFADGIPTIYSGQEQHYAGANDPYNREAIWLSGYATDSELYKFIATANEIRKLAISKDSSYLTTRNNAFYTDSNTIAMRKGTSGSQVITVLSNSGSSGGSYTLNLNNHGYSSGAQLVELYTCASVQVDSSGNMPVPMASGLPRVLVPGSWATGSGLCGTSSGTPSKTTTLITTTSQVSSSTSSTCVAATSLPIAFTEKVTTSYGESVFITGSISQLGNWNAANAVALSASQYTSANPVWTVSLDLPVGTTFQYKYIKKEQDGSVVWESDPNRSYTVSSGCTGVKQAVSDSWR

SEQ ID NO: 27 - protein, 590 aa, Penicillium funiculosum
LTADEWRSQSIYFLLTDRFGLTSNSTTASCDVADGLYCGGSWQGVINHLDYIQGMGFTAIWITPVTENFEGDTSDGEAYHGYWQQNAYATNSHYGASSDLLKLSEALHARGMYLMVDIVVNNMAYDGAGTSVDYSIFNPFPSESYYHSYCLINYNTYNATDWDDCWEGDTIVSLPDLDTTQTYVKDTWNTWVKSFVANYSIDGLRIDSALHIQQDFFTAFEEAAGVYCIGELDYGDPAVVCPYQSVLSGVLNYPIYWQLLYAFESSSGSISNLYNMINTVKSDCADTSLLGNFIENHDNPRFAYYTSDYSEAKNVISFIFLTDGIPILYYGQEQHYSGGNIPLNREPLWTSDYSTDAQLYTYTKTSNAIRSLAIAKDSAYLTYQNYPIYQDSNTIAMRKGTTGLQLVTVLSNLGANGSSYTLTLSGSGYTSGTVVTELYTCTNVTVSSSGTIAVPMASGSPRAFLPWSSVSGSSLCNSVSSGCTAASTVAVTFEEVVTTTYGQEVYLTGSISQLGSWSTSSAVLLSAAQYTSSDPVWTVTVNLPAGESFEYKFIIVNSDGTVTWESDPNRSYTVPTGCQGLTATVDDTWR

SEQ ID NO: 28 - protein, 603 aa, Aureobasidium pullulans
LTPAQWRSQSIYQVLTDRFARTDGSTTASCDVNKYCGGSFQGIIKKLDYIQQMGFTAIWISPVVKNIYSSGQDGDSYHGYWAQDIYQVNTNFGSAADLVSLSKALHDRGMYLMVDIVTNHMGYNGCGNCVDYSIYNPFNSQSYYHPFCLINYNDQTSVEQCWAGDNTVSLPDLRTEDSNVLSMWNTWIKQLVFNYTIDGLRIDSAKSVDKAFYQPFQQAASVYAVGEVYDGDPNYFCDYQNYLDGMLNYPTYYWITQAFQSTSGSISNLYNGINTMKSTCKDTTLLGSFMENHDVARFASLTSDYALAKNAIAFTMLADGIPIIYQGQEQHFSGSSVPNNREALWLSGYPTSSQLYPFIATVNKIRKQAIKQDTGYLTYKAYPVYSDASTIVMRKGTTGSQVIGVFTNKGSSGSSSFTLSSSASGFTAGQAVTDVLSCTSYTADSNGNIAININAGAPRVLYPTSKLTGSGLCSGSSSTSGTPTTIKTSAVSGGCSTPTAVAVTFTDKVTTQYGQTIKLAGSIPQLGSWNAANAVTLSSAGYTASNPVWSGTVNIPAGQAFSYKFIKVNSDGSVTWESDPNHSYTVPASCGVTTASVSNTWQG

SEQ ID NO: 29 - protein, 624 aa, Lipomyces starkeyi
YILRRDCTTVTVLSSPESVTSSNHVQLASHEMCDSTLSASLYIYNDDYDKIVTLYYLTSSGTTGSVTASYSSSLSNNWELWSLSAPAADAVEITGASYVDSDASATYATSFDIPLTTTTTSSSSASATSTSSLTTTSSVSISVSVPTGTAANWRGRAIYQIVTDRFARTDGSTTYLCDVTDRVYCGGSYQGIINMLDYIQGMGFTAIWISPIVENIPDDTGYGYAYHGYWMKDIFALNTNFGTADDLIALATELHNRGMYLMVDIVVNHFAFSGSHADVDYSEYFPYSSQDYFHSFCWITDYSNQTNVEQCWLGDDTVPLVDVNTQLDTVKSEYQSWVQELIANYSIDGLRIDTVKHVQMDFWAPFQEAAGIYAVGEVFDGDPSYTCPYQENLDGVLNYPVYYPVVSAFESVSGSVSSLVDMIDTLKSECTDTTLLGSFLENQDNPRFPSYTSDESLIKNAIAFTMLSDGIPIIYYGQEQGLNGGNDPYNREALWLTGYSTTSTFYKYIASLNQIRNQAIYKDDTYLTYQNWVIYSDSTTIAMRKGFTGNQIITVLSNLGTSGSSYTLTLSNTGYTASSVVYEILTCTAVTVDSSGNLAVPMSSGLPKVFYQESQLVGSGICSM

SEQ ID NO: 30 - protein, 422 aa, Oryza sativa
DKILFQGFNWESWRQSGGWYNLLMGKVDDIVAAGVTHVWLPPPSHSVSTQGYMPGRLYDLDASRYGTSMELKSLISALHGKGIQAIADVVINHRCADYKDSRGIYCIFEGGTPDGRLDWGPHMICRDDTQFSDGTGNLDTGADFAAAPDIDHLNGVVQRELTDWLLWLKSDEVGFDAWRLDFARGYSPEVAKVYIEGTTPVGLAVAELWDSMAYGGDGKPEYNQDAHRQALVDWVDRVGGTASAGMVFDFTTKGIMNTAVEGELWRLIDQQGKAPGVIGWWPAKAVTFVDNHDTGSTQQMWPFPSDKVMQGYAYILTHPGNPCIFYDHFFDWGLKEQIAALVAVRQRNGVTATSSLKIMLHDADAYVAEIDGKVVMKIGSRYDVSSLIPPGFHLAAHGNGYAVWEKSAAAAADHRTSSSASL

SEQ ID NO: 31 - protein, 615 aa, Aspergillus aculeatus
AEWRTQSIYFLLTDRFGRTDNSTTATCNTGDQVYCGGTWQGIINHLDYIQGMGFTAVWISPVTEQLSANTADGESYHGYWQQKIYSLNSNFGTADDLKALSAALHERDMYLMVDVVPNHMGYAGSGDSVDYSVFDAFDSSSYFHSYCLITDWDDIDQVRTCWEGDTIVSLPDLYTTQSDVRTIWYDWIEQLVANYSIDGLRIDSALEVEPDFFTGYVSAAGVYSVGEIFNGDPATACPYQGYLDGVLNYPIYFQLLYAFESSSGSISDLYNMINSVASDCSDPTLLGNFIENHDNARFAYYTSDYSQAKNVLSFLFLSDGIPIVYAGEEQHYSGSGVPYNREATWLSGYSTTAELYQWIATTNAIRKLAISLDSNYITYKNNPFYTDSNTIAMRKGSDNLQVITILSNRGSSSSSYTLTLTGTGYAAGTTLIEAYTCTTLTVSSSGSIAVPMASGLPRVYLPASSVNKGSLCGGGTSATTATTTTTLKTTTTTTSTKTTTTSCTATTTSLPITFIELVTTTYGEEIYLTGSIAALGNWATTASGRIALSAANYSASYPEWSATVSVPVGTSFEYKFFKVGTDGSTITWESDPNRVYTVTATACAGATATVVDSWR

SEQ ID NO: 32 - protein, 590 aa, Talaromyces leycettanus
LAPAEWRKQSIYFLLTDRFGRTDNSTTATCNVSDRVYCGGSWQGIINHLDYIQGMGFTAVWISPVTEQLPQDTGDGAAYHGYWQQRIYELNANFGTESDLKALATALHDRGMYLMLDVVANHMGYAGAGNTVDYSVFDPFDSSSYFHPYCLISDYSNQTNVEDCWLGDTTVSLPDLNTTETAVQNIWYNWVAGLVANYSVDGLRIDTVKHVQKPFWPGYNKAAGVYCVGEVLNGDPSYTCDYQNYLDAVLNYPIYFQLLYAFESSSGSIANLYNMINSVASVCVDPTLLGNFIENHDNPRFAYYTSDYSQAKNVIAYIFLADGIPIVYAGQEQHYSGGNDPYNREATWLSGYSTSAELYTFIATTNQIRKLAISRDSNYLTSRNNPFYYDSNTLAMRKGSSGSQVITVLSNLGSSGSSYTLTLSNTGYSSGTSLTELHTCTSVTVDSSGNIAVPMASGSPRVLVPSSWINGSGLCSGSGTTGCTAATSVPVLFEETVTTTYGENIFISGSISQLGDWDTSQAVALSASQYTASDPLWEVTIDLPVGTSFEYKFIKVEPSGTVVWESDPNRQYTVPTACTGTTETVVATWR

SEQ ID NO: 33 - protein, 464 aa, Thermoascus aurantiacus
ATPAQWRSRSVYFLLTDRFARSDGSTTAACDTSARLDYIQGMGFTAIWISPVTEQLPQDTGDGTAYHGYWQQDIYSLNPNFGTADDLRALADALHARGMYLMVDVVANHMGYAGPGNSVDYSVFNPFNKQEYFHPYCEITNYDDQSNVEDCWLGDTIVSLPDLNTTRSDVEDIWYSWVRALVSNYSVDGLRIDTVKHVQKDFWPGYNDAAGVYCVGEVFDGDPSYTCDYQNYLDGVLNYPMYYPLLRAFSSTSGSISDLYNMINTVKAQCADSTLLGTFVENHDVPRFASYTSDIALAKNAIAFTILSDGIPIIYAGQEQHYSGGNDPANREAVWLSGYSTTSELYQFIAVSNQIRNYAIYVDEGYLTYKAWPIYQDSHTLAIRKGFDGNQVITVLSNLGSSGSSYTLSLSGTGYAAGQQVTEIYSCTDVTADSNGNIAVSMGGGLPKAFFPTAKLAGSGICWK

SEQ ID NO: 34 - protein, 633 aa, Brevibacterium halotolerans
GPAAANAETQNTSNELTAPSIKSGTILHAWNWSFNTLKHNMKDIHDAGYTAIQTSPINQVKEGNQGNKSMSNWYWLYQPTSYQIGNRYLGTEQEFKEMCAAAEEYGVKVIVDAVINHTTSDYAAISNEIKSIPNWTHGNTQIKNWSDRWDVTQNSLLGLYDWNTQNTQVQSYLKRFLERALNDGADGFRYDAAKHIELPDDGNYGSQFWPNITNTSAEFQYGEILQDSASRDAAYANYMNVTASNYGHSIRSALKNRNLSVSNISHYASEVSADKLVTWVESHDTYANDEEESTWMSDDDIRLGWAVIASRSGSTPLFFSRPEGGGNGVRFPGKSQIGDRGSALFEDQAITAVNRFHNVMDGQPEELSNPNGNNQIFMNQRGSHGVVLANAGSSSVTINTSTKLPDGRYDNKAGNGSFQVTDGKLTGTINARSVAVLYSDDIANAPHVFLENVKTGVTHSFNDQLTITLRADANTTKAVYQINNGQETVFKDGDQLTIGKGDPFGTTYTITLTGTNSDGVTRTQEYSFVKREPSAAKTIGYQNPNHWGQVNAYIYKHDGGRALELTGSWPGKAMIKNADGIYTLTLPADTDTTNAKVIFNNGSAQVPGQNQPGFDYVQNGLYNDSGLSGSLPH